European Patent Specification EP 3 714 044 B1, published January 1, 2025. Title: Compositions and Methods for Enhancing Production, Growth, Spread, or Oncolytic and Immunotherapeutic Efficacy of Interferon-Sensitive Viruses. Applicant: Ottawa Hospital Research Institute University of Ottawa. The sequence listing filed with the application follows.

SEQUENCE LISTING (8 sequences)

SEQ ID NO: 1 - DNA, 20 bp, Artificial Sequence
  gapdh primer
acagtcagccgcatcttctt

SEQ ID NO: 2 - DNA, 20 bp, Artificial Sequence
  gapdh primer
gttaaaagcagccctggtga

SEQ ID NO: 3 - DNA, 20 bp, Artificial Sequence
  hmox1 primer
actgcgttcctgctcaacat

SEQ ID NO: 4 - DNA, 20 bp, Artificial Sequence
  hmox1 primer
ggggcagaatcttgcacttt

SEQ ID NO: 5 - DNA, 20 bp, Artificial Sequence
  nrf2 primer
caactactcccaggttgccc

SEQ ID NO: 6 - DNA, 20 bp, Artificial Sequence
  nrf2 primer
agtgactgaaacgtagccga

SEQ ID NO: 7 - DNA, 20 bp, Artificial Sequence
  ifitm1 primer
ccgtgaagtctagggacagg

SEQ ID NO: 8 - DNA, 20 bp, Artificial Sequence
  ifitm1 primer
ggtagactgtcacagagccg